European Patent Application EP 4 230 739 A1, published August 23, 2023. Title: MODIFIED PLANT ENDOSPERM SPECIFIC PROMOTER AND USE THEREOF. Applicant: WUHAN HEALTHGEN BIOTECHNOLOGY CORP. The sequence listing filed with the application follows.

SEQUENCE LISTING (10 sequences)

SEQ ID NO: 1 - DNA, 930 bp, Artificial Sequence
  Gt13aΔ281
tgaaacaatattatgagtaatgtgtgagcattatgggaccacgaaataaaaaaagaacatttttatgagcagtgtgttctcaatgagccttgaatgttatcacccaggataagaaacccttaagcaatgaaacatgcaagcgtttaatgtgcaaagttggcattctccacgacataatgcaaaagaagatataatctatgacatagcaagtcatgcatcatttcatgcctctgtcaacctattcatttctagtcatctaggtaagtatcttaagctaaagtgttagaacttcccatacataagtcataactgatgacaattgggtgtaacacatgacaaaccagagagtcaagcaagataaagcaaaaggatgtgtacataaaactacagagctatatgtcatgttgcgaaaagaggagagcttataagacaagccatgactcaaaaaaaattcacatgcctactgtggcccatatatcatgcaacaatccaaaaactcacaggtctcggtgttgatcgtgtcaacatgtgaccaccctaaaaactcttcactaaatattaaagtattgctagaacagagcttcaagatataagtcatgatcaccaacaaccatgttcaaaaagaaatagaaagctatggcacagcaacaaaaagcaaaagcatgcatggatataatctttaacatcatccatgtcatattgcaaaagaaagaaagagagaacaatacaaatgatgtgtcaattacacatccatcattatccatccaccttccgtgtaccacacttcatatatcatgagtcacttcatgtctggacattaacaaactctatcttaacattcaaatgcatgagactttatctcactataaatgcacaatgatttagcattgtttctcacaaaaccattcaagttcattagtactacaacaa

SEQ ID NO: 2 - DNA, 930 bp, Artificial Sequence
  Gt13aΔ281+AT
tgaaacaatattatgagtaatgtgtgagcattatgggaccacgaaataaaaaaagaacatttttatgagcagtgtgttctcaatgagccttgaatgttatcacccaggataagaaacccttaagcaatgaaacatgcaagcgtttaatgtgcaaagttggcattctccacgacataatgcaaaagaagatataatctatgacatagcaagtcatgcatcatttcatgcctctgtcaacctattcatttctagtcatctaggtaagtatcttaagctaaagtgttagaacttcccatacataagtcataactgatgacaatttggtgtaacacatgacaaaccagagagtcaagcaagataaagcaaaaggatgtgtacataaaactacagagctatatgtcatgttgcgaaaagaggagagcttataagacaagccatgactcaaaaaaaattcacatgcctactgtggcccatatatcatgcaacaatccaaaaactcacaggtctcggtgttgatcgtgtcaacatgtgaccaccctaaaaactcttcactaaatattaaagtattgctagaacagagcttcaagatataagtcatgatcaccaacaaccatgttcaaaaagaaatagaaagctatggcacagcaacaaaaagcaaaagcatgcatggatataatctttaacatcatccatgtcatattgcaaaataaataaagagagaacaatacaaatgatatgtcaattacacatccatcattatccatccaccttccgtgtaccacacttcatatatcatgagtcacttcatgtctggacattaacaaactctatcttaacattcaaatgcatgagactttatctcactataaatgcacaatgatttagcattgtttctcacaaaaccattcaagttcattagtactacaacaa

SEQ ID NO: 3 - DNA, 952 bp, Artificial Sequence
  Gt13aΔ281+CAAT
tgaaacaatattatgagtaatgtgtgagcattatgggaccacgaaataaaaaaagaacatttttatgagcagtgtgttctcaatgagccttgaatgttatcacccaggataagaaacccttaagcaatgaaacatgcaagcgtttaatgtgcaaagttggcattctccacgacataatgcaaaagaagatataatctatgacatagcaagtcatgcatcatttcatgcctctgtcaacctattcatttctagtcatctaggtaagtatcttaagctaaagtgttagaacttcccatacataagtcataactgatgacaattgggtgtaacacatgaccaatacaaatgatgtgtcaattacacatgagagtcaagcaagataaagcaaaaggatgtgtacataaaactacagagctatatgtcatgttgcgaaaagaggagagcttataagacaagccatgactcaaaaaaaattcacatgcctactgtggcccatatatcatgcaacaatccaaaaactcacaggtctcggtgttgatcgtgtcaatatgtgaccaccctaaaaactcttcactaaatattaaagtattgctagaacagagcttcaagatataagtcatgatcaccaacaattatgttcaaaaagaaatagaaagctatggcacagcaacaaaaagcaaaagcatgcatggatataatctttaacatcatccatgtcatattgcaaaagaaagaaagagagaacaatacaaatgatgtgtcaattacacatccatcattatccatccaccttccgtgtaccacacttcatatatcatgagtcacttcatgtctggacattaacaaactctatcttaacattcaaatgcatgagactttatctcactataaatgcacaatgatttagcattgtttctcacaaaaccattcaagttcattagtactacaacaa

SEQ ID NO: 4 - DNA, 910 bp, Artificial Sequence
  Gt13aΔ281/Del
tgaaacaatattatgagtaatgtgtgagcattatgggaccacgaaataaaaaaagaacatttttatgagcagtgtgttctcaatgagccttgaatgttatcacccaggataagaaacccttaagcaatgaaacatgcaagcgtttaatgtgcaaagttggcattctccacgacataatgcaaaagaagatataatctatgacatagcaagtcatgcatcatttcatgcctctgtcaacctattcatttctagtcatctaggtaagtatcttaagctaaagtgttagaacttcccatacatgacaatttggtgtaacacatgacaaaccagagagtcaagcaagataaagcaaaaggatgtgtacataaaactacagagctatatgtcatgttgcgaaaagaggagagcttataagacaagccatgactcaaaaaaaattcacatgcctactgtggcccatatatcatgcaacaatccaaaaactcacaggtctcggtgttgatcgtgtcaaaccaccctaaaaactcttcactaaatattaaagtattgctagaacagagcttcaagatataagtcatgatcaccaacaaccatgttcaaaaagaaatagaaagctatggcacagcaacaaaaagcaaaagcatgcatggatataatctttaacatcatccatgtcatattgcaaaacaattaaagagagaacaatacaaatgatgtgtcaattacacatccatcattatccatccaccttccgtgtaccacacttcatatatcatgagtcacttcatgtctggacattaacaaactctatcttaacattcaaatgcatgagactttatctcactataaatgcacaatgatttagcattgtttctcacaaaaccattcaagttcattagtactacaacaa

SEQ ID NO: 5 - DNA, 970 bp, Artificial Sequence
  Gt13aΔ281+GCN4
tgaaacaatattatgagtaatgtgtgagcattatgggaccacgaaataaaaaaagaacatttttatgagcagtgtgttctcaatgagccttgaatgttatcacccaggataagaaacccttaagcaatgaaacatgcaagcgtttaatgtgcaaagttggcattctccacgacataatgcaaaagaagatataatctatgacatagcaagtcatgcatcatttcatgcctctgtcaacctattcatttctagtcatctaggtaagtatcttaagctaaagtgttagaacttcccatacataagtcataactgatgacaattgggtgtaacacatgacaaaccagagagtcaagcaagataaagcaaaaggatgtgtacataaaactacagagctatatgtcatgttgcgaaaagaggagagcttataagacaagccatgactcaaaaaaaattcacatgcctactgtggcccatatatcatgcaacaatccaaaaactcacaggtctcggtgttgatcgtgtcaacatgtgaccaccctaaaaactcttcactaaatattaaagtattgctagaacagagcttcaagatataagtcatgatcaccaacaaccatgttcaaaaagaaatagaaagctatggcacagcaacaaaaagcaaaagcatgcatggatataatctttaacatcatccatgtcatattgcaaaagaaagaaagagagaacaatacaaatgatgtgtcaattacacatccatcattatccatccaccttccgtgtaccacacttcatatatcatgagtcacttcatatatcatgagtcacttcatgtctggacattaacaaactctatcttaacattaacaaactctatcttaacattcaaatgcatgagactttatctcactataaatgcacaatgatttagcattgtttctcacaaaaccattcaagttcattagtactacaacaa

SEQ ID NO: 6 - DNA, 1211 bp, Oryza sativa
tcacaccttatgtaaagtatttgttgcaagaaaagtctaagatgacagcaacctgctgagaagaacaactgacgatgtcataaggagagggagcttttcgataggtgccgtgcagttcaaagagttagttagcagtaggatgaagatttttgcacatggcaatgagaagttaattatggtgtaggcaacccaaatgaaacaccaaaatatgcacaagacagtttgttgtattctgtagtacagaataaactaaagtaatgaaagaagatggtgttagaaaatgaaacaatattatgagtaatgtgtgagcattatgggaccacgaaataaaaaaagaacatttttatgagcagtgtgttctcaatgagccttgaatgttatcacccaggataagaaacccttaagcaatgaaacatgcaagcgtttaatgtgcaaagttggcattctccacgacataatgcaaaagaagatataatctatgacatagcaagtcatgcatcatttcatgcctctgtcaacctattcatttctagtcatctaggtaagtatcttaagctaaagtgttagaacttcccatacataagtcataactgatgacaattgggtgtaacacatgacaaaccagagagtcaagcaagataaagcaaaaggatgtgtacataaaactacagagctatatgtcatgttgcgaaaagaggagagcttataagacaagccatgactcaaaaaaaattcacatgcctactgtggcccatatatcatgcaacaatccaaaaactcacaggtctcggtgttgatcgtgtcaacatgtgaccaccctaaaaactcttcactaaatattaaagtattgctagaacagagcttcaagatataagtcatgatcaccaacaaccatgttcaaaaagaaatagaaagctatggcacagcaacaaaaagcaaaagcatgcatggatataatctttaacatcatccatgtcatattgcaaaagaaagaaagagagaacaatacaaatgatgtgtcaattacacatccatcattatccatccaccttccgtgtaccacacttcatatatcatgagtcacttcatgtctggacattaacaaactctatcttaacattcaaatgcatgagactttatctcactataaatgcacaatgatttagcattgtttctcacaaaaccattcaagttcattagtactacaacaa

SEQ ID NO: 7 - DNA, 1772 bp, Artificial Sequence
  FSA
gagtctagcggaggcccaccagagcgagatcgcccaccgcttcaacgacctcggcgaggagcacttccgcggcctcgtgctcgtggccttcagccagtacctccagcagtgcccgttcgaggaccacgtgaagctcgtgaacgaggtgaccgagttcgccaagggctgcgtggccgaccagagcgccgccaactgcgagaagagcctccacgagctcctcggcgacaagctctgcaccgtggccagcctccgcgacaagtacggcgagatggccgactgctgcgagaagaaggagccggagcgcaacgagtgcttcctccagcacaaggacgacaacccgggcttcggccagctcgtgaccccggaggccgacgccatgtgcaccgccttccacgagaacgagcagcgcttcctcggcaagtacctctacgagatcgcccgccgccacccgtacttctacgccccggagctcctctactacgccgaggagtacaagggcgtgttcaccgagtgctgcgaggccgccgacaaggccgcctgcctcaccccgaaggtggacgccctccgcgagaaggtgctcgccagcagcgccaaggagcgcctcaagtgcgccagcctccagaagttcggcgagcgcgccttcaaggcctggagcgtggcccgcctcagccagaagttcccgaaggccgagttcgccgagatcagcaagctcgtgaccgacctcgccaagatccacaaggagtgctgccacggcgacctcctagagtgcgccgacgaccgcgccgacctcgccaagtacatctgcgagaaccaggacagcatcagcaccaagctcaaggagtgctgcggcaagccggtgctagagaagagccactgcatcagcgaggtggagcgcgacgagctcccggccgacctcccgccgctcgccgtggacttcgtggaggacaaggaggtgtgcaagaactaccaggaggccaaggacgtgttcctcggcaccttcctctacgagtacagccgccgccacccggagtacagcgtgagcctcctcctccgcctcgccaaggagtacgaggccaccctagagaagtgctgcgccaccgacgacccgccggcctgctacgcccacgtgttcgacgagttcaagccgctcgtggaggagccgcacaacctcgtgaagaccaactgcgagctcttcgagaagctcggcgagtacggcttccagaacgccctcctcgtgcgctacaccaagaaggtgccgcaggtgagcaccccgaccctcgtggaggtgagccgcagcctcggcaaggtgggcagcaagtgctgcacccacccggaggccgagcgcctcagctgcgccgaggactacctcagcgtggtgctcaaccgcctctgcgtgctccacgagaagaccccggtgagcgagcgcgtgaccaagtgctgcaccgagagcctcgtgaaccgccgcccgtgcttcagcgccctccaggtggacgagacctacgtgccgaaggagttcagcgccgagaccttcaccttccacgccgacctctgcaccctcccggaggccgagaagcagatcaagaagcagagcgccctcgtggagctcctcaagcacaagccgaaggccaccgaggagcagctcaagaccgtgatgggcgacttcggcagcttcgtggacaagtgctgcgccgccgaggacaaggaggcctgcttcgccgaggagggcccgaagctcgtggccgccgcccaggccgccctcgcctgagctcgag

SEQ ID NO: 8 - protein, 584 aa, Felis Catus
  FSA Amino acid sequence
EAHQSEIAHRFNDLGEEHFRGLVLVAFSQYLQQCPFEDHVKLVNEVTEFAKGCVADQSAANCEKSLHELLGDKLCTVASLRDKYGEMADCCEKKEPERNECFLQHKDDNPGFGQLVTPEADAMCTAFHENEQRFLGKYLYEIARRHPYFYAPELLYYAEEYKGVFTECCEAADKAACLTPKVDALREKVLASSAKERLKCASLQKFGERAFKAWSVARLSQKFPKAEFAEISKLVTDLAKIHKECCHGDLLECADDRADLAKYICENQDSISTKLKECCGKPVLEKSHCISEVERDELPADLPPLAVDFVEDKEVCKNYQEAKDVFLGTFLYEYSRRHPEYSVSLLLRLAKEYEATLEKCCATDDPPACYAHVFDEFKPLVEEPHNLVKTNCELFEKLGEYGFQNALLVRYTKKVPQVSTPTLVEVSRSLGKVGSKCCTHPEAERLSCAEDYLSVVLNRLCVLHEKTPVSERVTKCCTESLVNRRPCFSALQVDETYVPKEFSAETFTFHADLCTLPEAEKQIKKQSALVELLKHKPKATEEQLKTVMGDFGSFVDKCCAAEDKEACFAEEGPKLVAAAQAALA

SEQ ID NO: 9 - DNA, 20 bp, Artificial Sequence
  Forward primer
agctaccagggcaacagcga

SEQ ID NO: 10 - DNA, 22 bp, Artificial Sequence
  Reverse primer
atctcgtagaggtacttgccga